European Patent Application EP 4 424 714 A1, published September 4, 2024. Title: CONDITION-CONTROLLED SPLICEABLE CHIMERIC ANTIGEN RECEPTOR MOLECULE AND USE THEREOF. Applicant: SHANGHAI SINOBAY BIOTECHNOLOGY CO., LTD. The sequence listing filed with the application follows.

SEQUENCE LISTING (11 sequences)

SEQ ID NO: 1 - protein, 617 aa, Artificial Sequence
  Antigen Recognition Unit
MALPVTALLLPLALLLHAARPDYKDDDDKEVQLVESGGGLVQPGGSLRLSCAASGFTFSGYGMSWVRQAPGKGLEWVATITSGGTYTYYPDSVKGRFTISRDNAKNSLYLQMNSLRAEDTAVYYCARSLAGNAMDYWGQGTLVTVSSGGGGSGGGGSGGGGSEIVLTQSPATLSLSPGERATLSCRASQTISDYLHWYQQKPGQAPRLLIKFASQSISGIPARFSGSGSGTDFTLTISSLEPEDFAVYYCQNGHGFPRTFGQGTKVEIKASIEVMYPPPYLDNEKSNGTIIHVKGKHLCPSPLFPGPSKPFWVLVVVGGVLACYSLLVTVAFIIFWVRSKRSRLLHSDYMNMTPRRPGPTRKHYQPYAPPRDFAAYRSRFSVVKRGRKKLLYIFKQPFMRPVQTTQEEDGCSCRFPEEEEGGCELTRSGYCLDLKTQVQTPQGMKEISNIQVGDLVLSNTGYNEVLNVFPKSKKKSYKITLEDGKEIICSEEHLFPTQTGEMNISGGLKEGMCLYVKETKITLSPQNFRIQKQETTLLKEKSTEKNSLAKSILAVKNHFIELRSKLSERFISHKNTESSATHFHRGSASEGRAVLTNKVVKDFMLQTLNDIDIRGSA

SEQ ID NO: 2 - protein, 763 aa, Artificial Sequence
  Antigen Recognition Unit
MALPVTALLLPLALLLHAARPDYKDDDDKEVQLVESGGGLVQPGGSLRLSCAASGFTFSGYGMSWVRQAPGKGLEWVATITSGGTYTYYPDSVKGRFTISRDNAKNSLYLQMNSLRAEDTAVYYCARSLAGNAMDYWGQGTLVTVSSGGGGSGGGGSGGGGSEIVLTQSPATLSLSPGERATLSCRASQTISDYLHWYQQKPGQAPRLLIKFASQSISGIPARFSGSGSGTDFTLTISSLEPEDFAVYYCQNGHGFPRTFGQGTKVEIKASIEVMYPPPYLDNEKSNGTIIHVKGKHLCPSPLFPGPSKPFWVLVVVGGVLACYSLLVTVAFIIFWVRSKRSRLLHSDYMNMTPRRPGPTRKHYQPYAPPRDFAAYRSRFSVVKRGRKKLLYIFKQPFMRPVQTTQEEDGCSCRFPEEEEGGCELTRSGYCLDLKTQVQTPQGMKEISNIQVGDLVLSNTGYNEVLNVFPKSKKKSYKITLEDGKEIICSEEHLFPTQTGEMNISGGLKEGMCLYVKESLALSLTADQMVSALLDAEPPILYSEYDPTRPFSEASMMGLLTNLADRELVHMINWAKRVPGFVDLALHDQVHLLECAWMEILMIGLVWRSMEHPGKLLFAPNLLLDRNQGKCVEGGVEIFDMLLATSSRFRMMNLQGEEFVCLKSIILLNSGVYTFLSSTLKSLEEKDHIHRVLDKITDTLIHLMAKAGLTLQQQHQRLAQLLLILSHIRHMSSKRMEHLYSMKCKNVVPLSDLLLEMLDAHRL

SEQ ID NO: 3 - protein, 379 aa, Artificial Sequence
  Signal Transduction Unit
MSEDTSSLFDKLKKEPDALTLLAPAAGDTIISLDFGSNDTETDDQQLEEVPLYNDVMLPSPNEKLQNINLAMSPLPTAETPKPLRSSADPALNQEVALKLEPNPESLELSFTMPQIQDQTPSPSDGSTRQSSPEPNSPSEYCFYVDSDMVNEFKLELVEKLFAEDTEAKNPFSTQDTDLDLEMLAPYIPMDDDFQLRSFDQLSPLESSSASPESASPQSTVTVFQLKKILKIEELDERELIDIEVSGNHLFYANDILTHNSSSSDVRVKFSRSADAPAYQQGQNQLYNELNLGRREEYDVLDKRRGRDPEMGGKPQRRKNPQEGLYNELQKDKMAEAYSEIGMKGERRRGKGHDGLYQGLSTATKDTYDALHMQALPPR

SEQ ID NO: 4 - DNA, 1453 bp, Artificial Sequence
  Signal Transduction Unit Containing A Hypoxia Response Element
ccacagtgcatacgtgggctccaacaggtcctcttccacagtgcatacgtgggctccaacaggtcctcttccacagtgcatacgtgggctccaacaggtcctcttccacagtgcatacgtgggctccaacaggtcctcttccacagtgcatacgtgggctccaacaggtcctcttaccaaaatcaacgggactttccaaaatgtcgtaacaactccgccccattgacgcaaatgggcggtaggcgtgtacggtgggaggtctatataagcagagctggtttagtgaaccgtcagatccgcttctagagccaccatgagcgaggacaccagcagcctgttcgacaagctgaagaaggagcccgacgccctgaccctgctggcccctgctgctggagacaccatcatctccctggacttcggcagcaacgacaccgagaccgacgaccagcagctggaggaggtgcccctgtacaacgacgtgatgctgccctctcccaacgaaaaactgcagaacatcaacctggctatgagccccctgcccaccgccgaaacaccaaaacccctgagatccagcgccgaccccgccctgaaccaggaagtggccctgaaactggaacccaaccccgagagcctggagctgagcttcaccatgccccagatccaggaccagacccccagccccagcgacggaagcaccagacagagcagccccgagcctaactcccccagcgaatactgcttctatgtggacagcgacatggtgaacgagttcaagctggagctggtggaaaaactgttcgccgaggacacagaagccaaaaaccccttcagcacccaggacacagacctggacctggagatgctggccccctacatccccatggacgacgacttccagctgagatccttcgaccagctgagccccctggaaagcagcagcgcctcccccgaatcagccagcccccagagcaccgtgaccgtgttccagctgaaaaagatcctgaagatcgaggagctggacgagcgggaactgatcgacatcgaagtgtccggaaaccacctgttctacgccaacgacatcctgacacacaatagcagcagcagcgacgtgagagtgaaattcagcagaagcgccgacgcccccgcctaccagcagggacagaatcagctgtacaacgaactgaacctgggcagaagggaggaatacgacgtgctggacaagaggagaggaagggaccccgagatgggaggaaaaccacagagaagaaagaacccacaggagggactgtacaacgagctgcagaaggacaagatggccgaggcctacagtgaaattggcatgaagggagagagaagaagaggaaagggacacgacggcctgtaccagggcctgagcaccgctaccaaggacacatacgacgccctgcacatgcaggccctgccaccaagatga

SEQ ID NO: 5 - DNA, 4673 bp, Artificial Sequence
  Condition-controlled Spliceable Chimeric Antigen Receptor
gctccggtgcccgtcagtgggcagagcgcacatcgcccacagtccccgagaagttggggggaggggtcggcaattgaaccggtgcctagagaaggtggcgcggggtaaactgggaaagtgatgtcgtgtactggctccgcctttttcccgagggtgggggagaaccgtatataagtgcagtagtcgccgtgaacgttctttttcgcaacgggtttgccgccagaacacaggtaagtgccgtgtgtggttcccgcgggcctggcctctttacgggttatggcccttgcgtgccttgaattacttccacgcccctggctgcagtacgtgattcttgatcccgagcttcgggttggaagtgggtgggagagttcgaggccttgcgcttaaggagccccttcgcctcgtgcttgagttgaggcctggcttgggcgctggggccgccgcgtgcgaatctggtggcaccttcgcgcctgtctccctgctttcgataagtctctagccatttaaaatttttgatgacctgctgcgacgctttttttctggcaagatagtcttgtaaatgcgggccaagatctgcacactggtatttcggtttttggggccgcgggcggcgacggggcccgtgcgtcccagcgcacatgttcggcgaggcggggcctgcgagcgcggccaccgagaatcggacgggggtagtctcaagctggccggcctgctctggtgcctggcctcgcgccgccgtgtatcgccccgccctgggcggcaaggctggcccggtcggcaccagttgcgtgagcggaaagatggccgcttcccggccctgctgcagggagctcaaaatggaggacgcggcgctcgggagagcgggcgggtgagtcacccacacaaaggaaaagggcctttccgtcctcagccgtcgcttcatgtgactccacggagtaccgggcgccgtccaggcacctcgattagttctcgagcttttggagtacgtcgtctttaggttggggggaggggttttatgcgatggagtttccccacactgagtgggtggagactgaagttaggccagcttggcacttgatgtaattctccttggaatttgccctttttgagtttggatcttggttcattctcaagcctcagacagtggttcaaagtttttttcttccatttcaggtgtcgtgaggatctatttccggtgagacccaagctggctagcgccaccatggctctgccagtgacagctctcctcctcccactcgccctgctgctgcacgccgctagacctgactacaaggacgacgacgacaaggaggtgcagctggtggagtctgggggaggcttggtccagcctggggggtccctgagactctcctgtgcagcctctggattcacctttagtggctatggcatgagctgggtccgccaggctccagggaaggggctggagtgggtggccaccataactagtggtggaacttacacctactatccagactctgtgaagggccgattcaccatctccagagacaacgccaagaactcactgtatctgcaaatgaacagcctgagagccgaggacacggctgtgtattactgtgcgagatccctcgcgggaaatgctatggactactggggccaaggaaccctggtcaccgtctcctcaggcggaggcggcagtggcgggggcgggtccggcggaggcgggagcgaaattgtgttgacacagtctccagccaccctgtctttgtctccaggggaaagagccaccctctcctgcagggccagtcagactattagcgactacttacactggtaccaacagaaacctggccaggctcccaggctcctcatcaaatttgcatcccaatccatttctggcatcccagccaggttcagtggcagtgggtctgggacagacttcactctcaccatcagcagcctagagcctgaagattttgcagtttattactgtcagaatggtcacggctttcctcggacgttcggccaagggaccaaggtggaaatcaaagctagcatcgaggtgatgtaccctcccccttacctggacaacgagaagagcaacggcaccatcatccacgtgaagggcaagcacctgtgccctagccccctgttccccggacctagcaagcccttttgggtgctggtggtggtgggcggcgtgctggcctgttactccctgctggtgaccgtggccttcattatcttctgggtgaggagcaagaggagcaggctgctgcacagcgactacatgaacatgacacccaggagacctggccccaccagaaagcactaccagccctatgccccccccagagactttgccgcctacagaagcaggttcagcgtggtgaagaggggcaggaagaagctgctgtacatcttcaagcagcccttcatgaggcccgtgcagaccacccaggaggaggacggctgcagctgcaggttccccgaggaggaggaaggcggatgcgagctgacccggtctggctactgcctcgacctcaagacccaggtgcagacccctcagggcatgaaggagatttctaacattcaggtgggcgacctcgtgctgagcaacaccggctacaacgaggtgctcaacgtgttcccaaagtctaagaagaagtcttacaagatcacactggaggacggcaaggagattatttgctctgaggagcacctgttccctacccagacaggcgagatgaacatttctggcggcctcaaggagggcatgtgcctgtacgtgaaggagaccaagatcaccctgagcccccagaacttccgcatccagaagcaggagaccaccctgctgaaggagaagagcaccgagaagaacagcctggccaagagcatcctggccgtgaagaaccacttcatcgagctgcgcagcaagctgagcgagcgcttcatcagccacaagaacaccgagagcagcgccacccacttccaccgcggcagcgccagcgagggccgcgccgtgctgaccaacaaggtggtgaaggacttcatgctgcagaccctgaacgacatcgacatccgcggcagcgcctgaacgcgtaaatgtggtatggctgattatgatccgatatctccagtgtggtgtgcaggatcccagcacagtctccaggcgatctgacggttcactaaacgagctctgcttatataggcctcccaccgtacacgccacctcgacataccacagtgcatacgtgggctccaacaggtcctcttccacagtgcatacgtgggctccaacaggtcctcttccacagtgcatacgtgggctccaacaggtcctcttccacagtgcatacgtgggctccaacaggtcctcttccacagtgcatacgtgggctccaacaggtcctcttaccaaaatcaacgggactttccaaaatgtcgtaacaactccgccccattgacgcaaatgggcggtaggcgtgtacggtgggaggtctatataagcagagctggtttagtgaaccgtcagatccgcttctagagccaccatgagcgaggacaccagcagcctgttcgacaagctgaagaaggagcccgacgccctgaccctgctggcccctgctgctggagacaccatcatctccctggacttcggcagcaacgacaccgagaccgacgaccagcagctggaggaggtgcccctgtacaacgacgtgatgctgccctctcccaacgaaaaactgcagaacatcaacctggctatgagccccctgcccaccgccgaaacaccaaaacccctgagatccagcgccgaccccgccctgaaccaggaagtggccctgaaactggaacccaaccccgagagcctggagctgagcttcaccatgccccagatccaggaccagacccccagccccagcgacggaagcaccagacagagcagccccgagcctaactcccccagcgaatactgcttctatgtggacagcgacatggtgaacgagttcaagctggagctggtggaaaaactgttcgccgaggacacagaagccaaaaaccccttcagcacccaggacacagacctggacctggagatgctggccccctacatccccatggacgacgacttccagctgagatccttcgaccagctgagccccctggaaagcagcagcgcctcccccgaatcagccagcccccagagcaccgtgaccgtgttccagctgaaaaagatcctgaagatcgaggagctggacgagcgggaactgatcgacatcgaagtgtccggaaaccacctgttctacgccaacgacatcctgacacacaatagcagcagcagcgacgtgagagtgaaattcagcagaagcgccgacgcccccgcctaccagcagggacagaatcagctgtacaacgaactgaacctgggcagaagggaggaatacgacgtgctggacaagaggagaggaagggaccccgagatgggaggaaaaccacagagaagaaagaacccacaggagggactgtacaacgagctgcagaaggacaagatggccgaggcctacagtgaaattggcatgaagggagagagaagaagaggaaagggacacgacggcctgtaccagggcctgagcaccgctaccaaggacacatacgacgccctgcacatgcaggccctgccaccaagatga

SEQ ID NO: 6 - DNA, 4376 bp, Artificial Sequence
  Condition-controlled Spliceable Chimeric Antigen Receptor
gctccggtgcccgtcagtgggcagagcgcacatcgcccacagtccccgagaagttggggggaggggtcggcaattgaaccggtgcctagagaaggtggcgcggggtaaactgggaaagtgatgtcgtgtactggctccgcctttttcccgagggtgggggagaaccgtatataagtgcagtagtcgccgtgaacgttctttttcgcaacgggtttgccgccagaacacaggtaagtgccgtgtgtggttcccgcgggcctggcctctttacgggttatggcccttgcgtgccttgaattacttccacgcccctggctgcagtacgtgattcttgatcccgagcttcgggttggaagtgggtgggagagttcgaggccttgcgcttaaggagccccttcgcctcgtgcttgagttgaggcctggcttgggcgctggggccgccgcgtgcgaatctggtggcaccttcgcgcctgtctccctgctttcgataagtctctagccatttaaaatttttgatgacctgctgcgacgctttttttctggcaagatagtcttgtaaatgcgggccaagatctgcacactggtatttcggtttttggggccgcgggcggcgacggggcccgtgcgtcccagcgcacatgttcggcgaggcggggcctgcgagcgcggccaccgagaatcggacgggggtagtctcaagctggccggcctgctctggtgcctggcctcgcgccgccgtgtatcgccccgccctgggcggcaaggctggcccggtcggcaccagttgcgtgagcggaaagatggccgcttcccggccctgctgcagggagctcaaaatggaggacgcggcgctcgggagagcgggcgggtgagtcacccacacaaaggaaaagggcctttccgtcctcagccgtcgcttcatgtgactccacggagtaccgggcgccgtccaggcacctcgattagttctcgagcttttggagtacgtcgtctttaggttggggggaggggttttatgcgatggagtttccccacactgagtgggtggagactgaagttaggccagcttggcacttgatgtaattctccttggaatttgccctttttgagtttggatcttggttcattctcaagcctcagacagtggttcaaagtttttttcttccatttcaggtgtcgtgaggatctatttccggtgagacccaagctggctagcgccaccatggctctgccagtgacagctctcctcctcccactcgccctgctgctgcacgccgctagacctgactacaaggacgacgacgacaaggaggtgcagctggtggagtctgggggaggcttggtccagcctggggggtccctgagactctcctgtgcagcctctggattcacctttagtggctatggcatgagctgggtccgccaggctccagggaaggggctggagtgggtggccaccataactagtggtggaacttacacctactatccagactctgtgaagggccgattcaccatctccagagacaacgccaagaactcactgtatctgcaaatgaacagcctgagagccgaggacacggctgtgtattactgtgcgagatccctcgcgggaaatgctatggactactggggccaaggaaccctggtcaccgtctcctcaggcggaggcggcagtggcgggggcgggtccggcggaggcgggagcgaaattgtgttgacacagtctccagccaccctgtctttgtctccaggggaaagagccaccctctcctgcagggccagtcagactattagcgactacttacactggtaccaacagaaacctggccaggctcccaggctcctcatcaaatttgcatcccaatccatttctggcatcccagccaggttcagtggcagtgggtctgggacagacttcactctcaccatcagcagcctagagcctgaagattttgcagtttattactgtcagaatggtcacggctttcctcggacgttcggccaagggaccaaggtggaaatcaaagctagcatcgaggtgatgtaccctcccccttacctggacaacgagaagagcaacggcaccatcatccacgtgaagggcaagcacctgtgccctagccccctgttccccggacctagcaagcccttttgggtgctggtggtggtgggcggcgtgctggcctgttactccctgctggtgaccgtggccttcattatcttctgggtgaggagcaagaggagcaggctgctgcacagcgactacatgaacatgacacccaggagacctggccccaccagaaagcactaccagccctatgccccccccagagactttgccgcctacagaagcaggttcagcgtggtgaagaggggcaggaagaagctgctgtacatcttcaagcagcccttcatgaggcccgtgcagaccacccaggaggaggacggctgcagctgcaggttccccgaggaggaggaaggcggatgcgagctgacccggtctggctactgcctcgacctcaagacccaggtgcagacccctcagggcatgaaggagatttctaacattcaggtgggcgacctcgtgctgagcaacaccggctacaacgaggtgctcaacgtgttcccaaagtctaagaagaagtcttacaagatcacactggaggacggcaaggagattatttgctctgaggagcacctgttccctacccagacaggcgagatgaacatttctggcggcctcaaggagggcatgtgcctgtacgtgaaggagtgaacgcgtaaatgtggtatggctgattatgatccgatatctccagtgtggtgtgcaggatcccagcacagtctccaggcgatctgacggttcactaaacgagctctgcttatataggcctcccaccgtacacgccacctcgacataccacagtgcatacgtgggctccaacaggtcctcttccacagtgcatacgtgggctccaacaggtcctcttccacagtgcatacgtgggctccaacaggtcctcttccacagtgcatacgtgggctccaacaggtcctcttccacagtgcatacgtgggctccaacaggtcctcttaccaaaatcaacgggactttccaaaatgtcgtaacaactccgccccattgacgcaaatgggcggtaggcgtgtacggtgggaggtctatataagcagagctggtttagtgaaccgtcagatccgcttctagagccaccatgagcgaggacaccagcagcctgttcgacaagctgaagaaggagcccgacgccctgaccctgctggcccctgctgctggagacaccatcatctccctggacttcggcagcaacgacaccgagaccgacgaccagcagctggaggaggtgcccctgtacaacgacgtgatgctgccctctcccaacgaaaaactgcagaacatcaacctggctatgagccccctgcccaccgccgaaacaccaaaacccctgagatccagcgccgaccccgccctgaaccaggaagtggccctgaaactggaacccaaccccgagagcctggagctgagcttcaccatgccccagatccaggaccagacccccagccccagcgacggaagcaccagacagagcagccccgagcctaactcccccagcgaatactgcttctatgtggacagcgacatggtgaacgagttcaagctggagctggtggaaaaactgttcgccgaggacacagaagccaaaaaccccttcagcacccaggacacagacctggacctggagatgctggccccctacatccccatggacgacgacttccagctgagatccttcgaccagctgagccccctggaaagcagcagcgcctcccccgaatcagccagcccccagagcaccgtgaccgtgttccagctgaaaaagatcctgaagatcgaggagctggacgagcgggaactgatcgacatcgaagtgtccggaaaccacctgttctacgccaacgacatcctgacacacaatagcagcagcagcgacgtgagagtgaaattcagcagaagcgccgacgcccccgcctaccagcagggacagaatcagctgtacaacgaactgaacctgggcagaagggaggaatacgacgtgctggacaagaggagaggaagggaccccgagatgggaggaaaaccacagagaagaaagaacccacaggagggactgtacaacgagctgcagaaggacaagatggccgaggcctacagtgaaattggcatgaagggagagagaagaagaggaaagggacacgacggcctgtaccagggcctgagcaccgctaccaaggacacatacgacgccctgcacatgcaggccctgccaccaagatga

SEQ ID NO: 7 - DNA, 1614 bp, Artificial Sequence
  CD47-28BBz
atggctctgccagtgacagctctcctcctcccactcgccctgctgctgcacgccgctagacctgactacaaggacgacgacgacaaggaggtgcagctggtggagtctgggggaggcttggtccagcctggggggtccctgagactctcctgtgcagcctctggattcacctttagtggctatggcatgagctgggtccgccaggctccagggaaggggctggagtgggtggccaccataactagtggtggaacttacacctactatccagactctgtgaagggccgattcaccatctccagagacaacgccaagaactcactgtatctgcaaatgaacagcctgagagccgaggacacggctgtgtattactgtgcgagatccctcgcgggaaatgctatggactactggggccaaggaaccctggtcaccgtctcctcaggcggaggcggcagtggcgggggcgggtccggcggaggcgggagcgaaattgtgttgacacagtctccagccaccctgtctttgtctccaggggaaagagccaccctctcctgcagggccagtcagactattagcgactacttacactggtaccaacagaaacctggccaggctcccaggctcctcatcaaatttgcatcccaatccatttctggcatcccagccaggttcagtggcagtgggtctgggacagacttcactctcaccatcagcagcctagagcctgaagattttgcagtttattactgtcagaatggtcacggctttcctcggacgttcggccaagggaccaaggtggaaatcaaagctagcatcgaggtgatgtaccctcccccttacctggacaacgagaagagcaacggcaccatcatccacgtgaagggcaagcacctgtgccctagccccctgttccccggacctagcaagcccttttgggtgctggtggtggtgggcggcgtgctggcctgttactccctgctggtgaccgtggccttcattatcttctgggtgaggagcaagaggagcaggctgctgcacagcgactacatgaacatgacacccaggagacctggccccaccagaaagcactaccagccctatgccccccccagagactttgccgcctacagaagcaggttcagcgtggtgaagaggggcaggaagaagctgctgtacatcttcaagcagcccttcatgaggcccgtgcagaccacccaggaggaggacggctgcagctgcaggttccccgaggaggaggaaggcggatgcgagctgagagtgaagttctccagaagcgctgacgcccctgcctaccagcagggacagaaccagctgtataacgagctgaacctgggcaggagagaggagtacgatgtcctggacaagaggagaggacgtgatcctgagatgggcggcaagccccaaaggagaaagaacccccaggagggactgtacaatgagctgcagaaggacaagatggccgaggcctactccgaaatcggcatgaaaggcgagaggagaaggggcaaaggccacgatggcctgtaccagggcctgagcacagccaccaaagacacatacgacgccctgcacatgcaggccctgccccctagg

SEQ ID NO: 8 - DNA, 2337 bp, Artificial Sequence
  CD47-28BBz-ODD
atggctctgccagtgacagctctcctcctcccactcgccctgctgctgcacgccgctagacctgactacaaggacgacgacgacaaggaggtgcagctggtggagtctgggggaggcttggtccagcctggggggtccctgagactctcctgtgcagcctctggattcacctttagtggctatggcatgagctgggtccgccaggctccagggaaggggctggagtgggtggccaccataactagtggtggaacttacacctactatccagactctgtgaagggccgattcaccatctccagagacaacgccaagaactcactgtatctgcaaatgaacagcctgagagccgaggacacggctgtgtattactgtgcgagatccctcgcgggaaatgctatggactactggggccaaggaaccctggtcaccgtctcctcaggcggaggcggcagtggcgggggcgggtccggcggaggcgggagcgaaattgtgttgacacagtctccagccaccctgtctttgtctccaggggaaagagccaccctctcctgcagggccagtcagactattagcgactacttacactggtaccaacagaaacctggccaggctcccaggctcctcatcaaatttgcatcccaatccatttctggcatcccagccaggttcagtggcagtgggtctgggacagacttcactctcaccatcagcagcctagagcctgaagattttgcagtttattactgtcagaatggtcacggctttcctcggacgttcggccaagggaccaaggtggaaatcaaagctagcatcgaggtgatgtaccctcccccttacctggacaacgagaagagcaacggcaccatcatccacgtgaagggcaagcacctgtgccctagccccctgttccccggacctagcaagcccttttgggtgctggtggtggtgggcggcgtgctggcctgttactccctgctggtgaccgtggccttcattatcttctgggtgaggagcaagaggagcaggctgctgcacagcgactacatgaacatgacacccaggagacctggccccaccagaaagcactaccagccctatgccccccccagagactttgccgcctacagaagcaggttcagcgtggtgaagaggggcaggaagaagctgctgtacatcttcaagcagcccttcatgaggcccgtgcagaccacccaggaggaggacggctgcagctgcaggttccccgaggaggaggaaggcggatgcgagctgagagtgaagttctccagaagcgctgacgcccctgcctaccagcagggacagaaccagctgtataacgagctgaacctgggcaggagagaggagtacgatgtcctggacaagaggagaggacgtgatcctgagatgggcggcaagccccaaaggagaaagaacccccaggagggactgtacaatgagctgcagaaggacaagatggccgaggcctactccgaaatcggcatgaaaggcgagaggagaaggggcaaaggccacgatggcctgtaccagggcctgagcacagccaccaaagacacatacgacgccctgcacatgcaggccctgccccctaggctcgagggcggaggcgggtccgggggcgggggctccggcggcggagggtccagcgaggatacctcatcactgtttgacaagctcaagaaggagcccgacgcactcacactcctcgcacccgccgccggcgatacaattattagcctggactttgggtctaacgatacagagaccgacgaccagcagctggaggaggtgcctctgtacaatgatgtcatgctgccttctcctaatgagaagctgcaaaatattaatctggctatgtcaccactgcctaccgccgagacacctaagccactcaggtctagcgccgatcccgctctgaaccaggaggtggccctgaagctagagccaaacccagagtctctggagctttcatttactatgccacagattcaggatcagactccatctccatccgacggatcaactaggcagtcttcccctgagcccaattccccatccgagtactgcttctacgtcgatagcgacatggtgaatgagtttaagctggagttagtcgagaagctgttcgcagaggatactgaggcaaagaacccattttcaacacaggacaccgacctggacttagaaatgctcgcaccttacattcctatggacgatgactttcagctgcggtcatttgatcagctgtcccctctcgaatcttctagcgcaagtcctgagagcgcttcaccacagtcaaccgtgaccgtgttccag

SEQ ID NO: 9 - DNA, 1854 bp, Artificial Sequence
  CD47-28BB-IntN-SopE
atggctctgccagtgacagctctcctcctcccactcgccctgctgctgcacgccgctagacctgactacaaggacgacgacgacaaggaggtgcagctggtggagtctgggggaggcttggtccagcctggggggtccctgagactctcctgtgcagcctctggattcacctttagtggctatggcatgagctgggtccgccaggctccagggaaggggctggagtgggtggccaccataactagtggtggaacttacacctactatccagactctgtgaagggccgattcaccatctccagagacaacgccaagaactcactgtatctgcaaatgaacagcctgagagccgaggacacggctgtgtattactgtgcgagatccctcgcgggaaatgctatggactactggggccaaggaaccctggtcaccgtctcctcaggcggaggcggcagtggcgggggcgggtccggcggaggcgggagcgaaattgtgttgacacagtctccagccaccctgtctttgtctccaggggaaagagccaccctctcctgcagggccagtcagactattagcgactacttacactggtaccaacagaaacctggccaggctcccaggctcctcatcaaatttgcatcccaatccatttctggcatcccagccaggttcagtggcagtgggtctgggacagacttcactctcaccatcagcagcctagagcctgaagattttgcagtttattactgtcagaatggtcacggctttcctcggacgttcggccaagggaccaaggtggaaatcaaagctagcatcgaggtgatgtaccctcccccttacctggacaacgagaagagcaacggcaccatcatccacgtgaagggcaagcacctgtgccctagccccctgttccccggacctagcaagcccttttgggtgctggtggtggtgggcggcgtgctggcctgttactccctgctggtgaccgtggccttcattatcttctgggtgaggagcaagaggagcaggctgctgcacagcgactacatgaacatgacacccaggagacctggccccaccagaaagcactaccagccctatgccccccccagagactttgccgcctacagaagcaggttcagcgtggtgaagaggggcaggaagaagctgctgtacatcttcaagcagcccttcatgaggcccgtgcagaccacccaggaggaggacggctgcagctgcaggttccccgaggaggaggaaggcggatgcgagctgacccggtctggctactgcctcgacctcaagacccaggtgcagacccctcagggcatgaaggagatttctaacattcaggtgggcgacctcgtgctgagcaacaccggctacaacgaggtgctcaacgtgttcccaaagtctaagaagaagtcttacaagatcacactggaggacggcaaggagattatttgctctgaggagcacctgttccctacccagacaggcgagatgaacatttctggcggcctcaaggagggcatgtgcctgtacgtgaaggagaccaagatcaccctgagcccccagaacttccgcatccagaagcaggagaccaccctgctgaaggagaagagcaccgagaagaacagcctggccaagagcatcctggccgtgaagaaccacttcatcgagctgcgcagcaagctgagcgagcgcttcatcagccacaagaacaccgagagcagcgccacccacttccaccgcggcagcgccagcgagggccgcgccgtgctgaccaacaaggtggtgaaggacttcatgctgcagaccctgaacgacatcgacatccgcggcagcgcctga

SEQ ID NO: 10 - DNA, 2292 bp, Artificial Sequence
  CD47-28BB-IntN-ERm
atggctctgccagtgacagctctcctcctcccactcgccctgctgctgcacgccgctagacctgactacaaggacgacgacgacaaggaggtgcagctggtggagtctgggggaggcttggtccagcctggggggtccctgagactctcctgtgcagcctctggattcacctttagtggctatggcatgagctgggtccgccaggctccagggaaggggctggagtgggtggccaccataactagtggtggaacttacacctactatccagactctgtgaagggccgattcaccatctccagagacaacgccaagaactcactgtatctgcaaatgaacagcctgagagccgaggacacggctgtgtattactgtgcgagatccctcgcgggaaatgctatggactactggggccaaggaaccctggtcaccgtctcctcaggcggaggcggcagtggcgggggcgggtccggcggaggcgggagcgaaattgtgttgacacagtctccagccaccctgtctttgtctccaggggaaagagccaccctctcctgcagggccagtcagactattagcgactacttacactggtaccaacagaaacctggccaggctcccaggctcctcatcaaatttgcatcccaatccatttctggcatcccagccaggttcagtggcagtgggtctgggacagacttcactctcaccatcagcagcctagagcctgaagattttgcagtttattactgtcagaatggtcacggctttcctcggacgttcggccaagggaccaaggtggaaatcaaagctagcatcgaggtgatgtaccctcccccttacctggacaacgagaagagcaacggcaccatcatccacgtgaagggcaagcacctgtgccctagccccctgttccccggacctagcaagcccttttgggtgctggtggtggtgggcggcgtgctggcctgttactccctgctggtgaccgtggccttcattatcttctgggtgaggagcaagaggagcaggctgctgcacagcgactacatgaacatgacacccaggagacctggccccaccagaaagcactaccagccctatgccccccccagagactttgccgcctacagaagcaggttcagcgtggtgaagaggggcaggaagaagctgctgtacatcttcaagcagcccttcatgaggcccgtgcagaccacccaggaggaggacggctgcagctgcaggttccccgaggaggaggaaggcggatgcgagctgacccggtctggctactgcctcgacctcaagacccaggtgcagacccctcagggcatgaaggagatttctaacattcaggtgggcgacctcgtgctgagcaacaccggctacaacgaggtgctcaacgtgttcccaaagtctaagaagaagtcttacaagatcacactggaggacggcaaggagattatttgctctgaggagcacctgttccctacccagacaggcgagatgaacatttctggcggcctcaaggagggcatgtgcctgtacgtgaaggagtctctggccctgtccctcacagccgaccagatggtgtccgccctcctggacgccgagccaccaattctgtactctgagtacgacccaacacgccctttcagcgaggcctctatgatgggcctcctcacaaacctcgccgaccgggagctggtgcacatgattaactgggccaagagagtgcccggcttcgtggacctcgccctgcacgaccaggtgcacctgctggagtgcgcctggatggagatcctcatgattggcctggtgtggcggtctatggagcacccaggcaagctgctgttcgcccctaacctcctgctcgaccgcaaccagggcaagtgcgtggagggcggcgtggagattttcgacatgctcctcgccacatctagccggttccggatgatgaacctccaaggcgaggagttcgtgtgcctgaagtctattattctgctcaactctggcgtgtacaccttcctgtcttctacactcaagtctctggaggagaaggaccacattcaccgcgtgctcgacaagattaccgacacactcattcacctgatggccaaggccggcctcacactgcaacagcagcaccagagactggcccagctgctcctgatcctgtcccacattaggcacatgtcttctaagcgcatggagcacctgtactctatgaagtgcaagaacgtggtgccactgtctgacctgctcctggaaatgctggacgcccaccggctgtga

SEQ ID NO: 11 - DNA, 1140 bp, Artificial Sequence
  ODD-IntC-CD3z
atgagcgaggacaccagcagcctgttcgacaagctgaagaaggagcccgacgccctgaccctgctggcccctgctgctggagacaccatcatctccctggacttcggcagcaacgacaccgagaccgacgaccagcagctggaggaggtgcccctgtacaacgacgtgatgctgccctctcccaacgaaaaactgcagaacatcaacctggctatgagccccctgcccaccgccgaaacaccaaaacccctgagatccagcgccgaccccgccctgaaccaggaagtggccctgaaactggaacccaaccccgagagcctggagctgagcttcaccatgccccagatccaggaccagacccccagccccagcgacggaagcaccagacagagcagccccgagcctaactcccccagcgaatactgcttctatgtggacagcgacatggtgaacgagttcaagctggagctggtggaaaaactgttcgccgaggacacagaagccaaaaaccccttcagcacccaggacacagacctggacctggagatgctggccccctacatccccatggacgacgacttccagctgagatccttcgaccagctgagccccctggaaagcagcagcgcctcccccgaatcagccagcccccagagcaccgtgaccgtgttccagctgaaaaagatcctgaagatcgaggagctggacgagcgggaactgatcgacatcgaagtgtccggaaaccacctgttctacgccaacgacatcctgacacacaatagcagcagcagcgacgtgagagtgaaattcagcagaagcgccgacgcccccgcctaccagcagggacagaatcagctgtacaacgaactgaacctgggcagaagggaggaatacgacgtgctggacaagaggagaggaagggaccccgagatgggaggaaaaccacagagaagaaagaacccacaggagggactgtacaacgagctgcagaaggacaagatggccgaggcctacagtgaaattggcatgaagggagagagaagaagaggaaagggacacgacggcctgtaccagggcctgagcaccgctaccaaggacacatacgacgccctgcacatgcaggccctgccaccaagatga